European Patent Application EP 4 163 390 A1, published April 12, 2023. Title: METHOD FOR ANALYZING TARGET NUCLEIC ACID FROM CELL. Applicant: TENK GENOMICS, INC. The sequence listing filed with the application follows.

SEQUENCE LISTING (17 sequences)

SEQ ID NO: 1 - DNA, 18 bp, Artificial Sequence
  T7 promoter subsequence
taatacgactcactatag

SEQ ID NO: 2 - DNA, 33 bp, Artificial Sequence
  Tn5MEA
tcgtcggcagcgtcagatgtgtataagagacag

SEQ ID NO: 3 - DNA, 34 bp, Artificial Sequence
  Tn5MEB
gtctcgtgggctcggagatgtgtataagagacag

SEQ ID NO: 4 - DNA, 19 bp, Artificial Sequence
  Tn5NTS
ctgtctcttatacacatct

SEQ ID NO: 5 - DNA, 41 bp, Artificial Sequence
  Top1 chain
  misc_feature (16)..(16): n = a, c, g or t
  misc_feature (17)..(17): n = a, c, g or t
  misc_feature (18)..(18): n = a, c, g or t
  misc_feature (19)..(19): n = a, c, g or t
  misc_feature (20)..(20): n = a, c, g or t
  misc_feature (21)..(21): n = a, c, g or t
  misc_feature (22)..(22): n = a, c, g or t
aggccagagcattcgnnnnnnnagatgtgtataagagacag

SEQ ID NO: 6 - DNA, 33 bp, Artificial Sequence
  PCR adapter
acactctttccctacacgacgctcttccgatct

SEQ ID NO: 7 - DNA, 15 bp, Artificial Sequence
  linking sequence 1
cgactcactacaggg

SEQ ID NO: 8 - DNA, 15 bp, Artificial Sequence
  linking sequence 2
tcggtgacacgatcg

SEQ ID NO: 9 - DNA, 30 bp, Artificial Sequence
  Microsphere second chain complementary sequence
cgaatgctctggcctctcaagcacgtggat

SEQ ID NO: 10 - DNA, 58 bp, Artificial Sequence
  Primer TrueseqD501 sequence
aatgatacggcgaccaccgagatctacactctttccctacacgacgctcttccgatct

SEQ ID NO: 11 - DNA, 47 bp, Artificial Sequence
  Primer N701 sequence
caagcagaagacggcatacgagatatcggctagtctcgtgggctcgg

SEQ ID NO: 12 - DNA, 15 bp, Artificial Sequence
  Ligation linking sequence
atccacgtgcttgag

SEQ ID NO: 13 - DNA, 52 bp, Artificial Sequence
  RT primer
  misc_feature (16)..(16): n = a, c, g or t
  misc_feature (17)..(17): n = a, c, g or t
  misc_feature (18)..(18): n = a, c, g or t
  misc_feature (19)..(19): n = a, c, g or t
  misc_feature (20)..(20): n = a, c, g or t
  misc_feature (21)..(21): n = a, c, g or t
  misc_feature (22)..(22): n = a, c, g or t
aggccagagcattcgnnnnnnntttttttttttttttttttttttttttttt

SEQ ID NO: 14 - DNA, 30 bp, Artificial Sequence
  TSO primer
  misc_feature (28)..(28): n = riboguanine
  misc_feature (29)..(29): n = riboguanine
  misc_feature (30)..(30): n = riboguanine
aagcagtggtatcaacgcagagtacatnnn

SEQ ID NO: 15 - DNA, 23 bp, Artificial Sequence
  ISPCR primer
aagcagtggtatcaacgcagagt

SEQ ID NO: 16 - DNA, 25 bp, Artificial Sequence
  lattice DNA1
acactctttccctacacgacgctct

SEQ ID NO: 17 - DNA, 24 bp, Artificial Sequence
  lattice DNA2
aaaaaaaaaaaaaaaaaaaaaaaa